European Patent Application EP 4 414 448 A1, published August 14, 2024. Title: 转氨酶突变体及其应用. Applicant: 凯莱英医药集团（天津）股份有限公司. The sequence listing filed with the application follows.

SEQUENCE LISTING (2 sequences)

SEQ ID NO: 1 - protein, 484 aa, Arthrobacter citreus
MGLTVQKINWEQVKEWDRKYLMRTFSTQNEYQPVPIESTEGDYLITPGGTRLLDFFNQLYCVNLGQKNQKVNAAIKEALDRYGFVWDTYATDYKAKAAKIIIEDILGDEDWPGKVRFVSTGSEAVETALNIARLYTNRPLVVTREHDYHGWTGGAATVTRLRSFRSGLVGENSESFSAQIPGSSCSSAVLMAPSSNTFQDSNGNYLKDENGELLSVKYTRRMIENYGPEQVAAVITEVSQGVGSTMPPYEYVPQIRKMTKELGVLWISDEVLTGFGRTGKWFGYQHYGVQPDIITMGKGLSSSSLPAGAVVVSKEIAAFMDKHRWESVSTYAGHPVAMAAVCANLEVMMEENLVEQAKNSGEYIRSKLELLQEKHKSIGNFDGYGLLWIVDIVNAKTKTPYVKLDRNFRHGMNPNQIPTQIIMEKALEKGVLIGGAMPNTMRIGASLNVSRGDIDKAMDALDYALDYLESGEWQQSLEHHHHHH

SEQ ID NO: 2 - DNA, 1455 bp, Arthrobacter citreus
atgggcctgaccgtacagaagatcaactgggaacaagtaaaggagtgggaccgcaagtacctgatgcgcactttttccactcagaacgaataccagccggtaccgattgaatctacggaaggtgattatctgatcaccccgggtggcacccgtctgctggacttcttcaaccaactgtattgcgttaacctgggccagaaaaaccagaaagtcaacgccgcgattaaagaggcactggaccgctacggcttcgtatgggacacttatgctaccgactacaaggcgaaagccgcgaaaatcattatcgaggatattctgggtgacgaggattggcctggtaaagttcgttttgttagcactggctccgaagccgtggaaaccgcgctgaatatcgcgcgtctgtataccaatcgtccgctggttgtgacccgtgaacacgactatcacggttggaccggcggcgctgcaaccgtcactcgtctgcgtagcttccgttctggtctggtgggtgaaaactccgaaagcttctctgctcagatcccgggttcttcttgtagctctgcagtcctgatggccccgtcttccaacaccttccaggactctaacggcaactacctgaaagacgaaaacggtgaactgctgtccgttaaatacacccgtcgcatgattgaaaactacggcccggagcaggtagccgcagtgattacggaagttagccagggtgttggttctacgatgccgccatacgaatatgttccacagatccgtaaaatgactaaagagctgggcgttctgtggatctccgacgaggtcctgaccggttttggtcgtaccggtaaatggttcggttaccagcattatggcgttcaaccagatatcattactatgggcaagggcctgtcttcttcctctctgccggcgggcgcagtagttgtgtccaaagaaatcgctgcgtttatggacaaacaccgctgggaatctgtttccacctacgcgggtcacccggtggcgatggcagctgtgtgcgctaacctggaagtgatgatggaagaaaacctggtggaacaagctaaaaatagcggcgaatacatccgtagcaaactggaactgctgcaggaaaagcataaaagcatcggcaacttcgacggttacggtctgctgtggattgttgatatcgtgaatgcgaaaactaaaaccccgtatgtcaaactggatcgcaacttccgccacggcatgaacccgaaccagatcccgacgcagattatcatggaaaaagctctggaaaaaggcgttctgatcggtggtgcaatgcctaacactatgcgtatcggcgcatctctgaacgtatctcgtggtgatatcgataaagctatggatgctctggattacgcgctggattacctggagtccggtgaatggcagcagagcctcgagcaccaccaccaccaccactga